European Patent Application EP 4 582 444 A1, published July 9, 2025. Title: 中和呼吸道合胞病毒的C-型单域抗体及应用. Applicant: 武汉班科生物技术有限公司. Application WO. The sequence listing filed with the application follows.

SEQUENCE LISTING (42 sequences)

SEQ ID NO: 1 - protein, 10 aa, synthetic construct
GYNPYDFPII

SEQ ID NO: 2 - protein, 10 aa, synthetic construct
GYNPYDFPIV

SEQ ID NO: 3 - protein, 9 aa, synthetic construct
DENSYNTDS

SEQ ID NO: 4 - protein, 9 aa, synthetic construct
DENSYNTDR

SEQ ID NO: 5 - protein, 9 aa, synthetic construct
EENSYNTDR

SEQ ID NO: 6 - protein, 16 aa, synthetic construct
AREGGSSGEWYYDLWG

SEQ ID NO: 7 - protein, 16 aa, synthetic construct
ARVGGSSGEWYYDLWG

SEQ ID NO: 8 - protein, 16 aa, synthetic construct
AREGGSSGEWYYNLWG

SEQ ID NO: 9 - protein, 16 aa, synthetic construct
AREGGSSGDWYYDLWG

SEQ ID NO: 10 - protein, 114 aa, synthetic construct
PSVLCLPPKPKDTLVISRTPEVTCVVSGYNPYDFPIIKFKWYVDGVEVDNAKVKPRDENSYNTDSVVSKLTVLHQDWLNGKEYKCKVSAREGGSSGEWYYDLWGPIECTISKAK

SEQ ID NO: 11 - protein, 114 aa, synthetic construct
PSVSCLPPKPKDTFVISRTPEVTCVVSGYNPYDFPIIKFKWYVDGVEVDNAKVKPRDENSYNTDSVVSKLTVLHQDWLNGKEYKCKVSAREGGSSGEWYYDLWGPIECTISKAK

SEQ ID NO: 12 - protein, 114 aa, synthetic construct
PSVLCLPPKPKDTLVISRTPEVTCVVSGYNPYDFPIIKFKWYVDGVEVDNAKVKPRDENSYNTDSVISKLTVLHQDWLNGKEYKCKVSAREGGSSGEWYYDLWGPIECTISKAK

SEQ ID NO: 13 - protein, 114 aa, synthetic construct
PSVSCLPPKPKDTFVISRTPEVTCVVSGYNPYDFPIIKFKWYVDGVEVDNAKVKPRDENSYNTDSVISKLTVLHQDWLNGKEYKCKVSAREGGSSGEWYYDLWGPIECTISKAK

SEQ ID NO: 14 - protein, 114 aa, synthetic construct
PSVLCLPPKPKDTLMISRTPEVTCVVSGYNPYDFPIVKFKWYVDGVEVHNAKTKPRDENSYNTDRVVSKLTVLHQDWLNGKEYKCKVSAREGGSSGEWYYDLWGPIECTISKAK

SEQ ID NO: 15 - protein, 114 aa, synthetic construct
PTVLCLPPKPKDTLMISRTPEVTCVVSGYNPYDFPIIKFKWYVDGVEVHNAKTKPRDENSYNTDRVVSKLTVLHQDWLNGREYKCKVSAREGGSSGEWYYDLWGPIECTISKAN

SEQ ID NO: 16 - protein, 114 aa, synthetic construct
PSVLCLPPKPKDTLMISRTPEVTCVVSGYNPYDFPIIKFKWYVDGVEVHNGKTKPRDENSYNTDRVVSKLTVLHQDWLNGKEYKCKVSAREGGSSGEWYYDLWGPIECTISKAK

SEQ ID NO: 17 - protein, 114 aa, synthetic construct
PSVLCLPPKPKDTLMISRTPEVTCVVSGYNPYDFPIIKFKWYVDGVEVHNAKTKPRDENSYNTDRVVSKLTVLHQDWLNGKEYKCKVSAREGGSSGEWYYDLWGPIECTISKAK

SEQ ID NO: 18 - protein, 114 aa, synthetic construct
PSVLCLPPKPKDTLMISRTPEVTCVVSGYNPYDFPIVKFKWYVDGVEVHNAKTKPRDENSYNTDRVVSKLTVLHQDWLNGKEYKCKVSARVGGSSGEWYYDLWGPIECTIAKAK

SEQ ID NO: 19 - protein, 114 aa, synthetic construct
PSILCLPPKPKDTLMISRTPEVTCVVFGYNPYDFPIVKFKWYVDGVEMHNAKTKPRDENSYNTDRVVSKLTVLHQDWLNGKEYKCKVSARVGGSSGEWYYDLWGPIECTISKAK

SEQ ID NO: 20 - protein, 114 aa, synthetic construct
PSVLCLPPKPNDTLMISRTPEVTCVVSGYNPYDFPIVKFKWYVDGEEVHNAKTKPREENSYNTDRVVSKLTVPHQDWLNGKEYKCKVSARVGGSSGEWYYDLWGPIECTISKAK

SEQ ID NO: 21 - protein, 114 aa, synthetic construct
PSVLCLPPKPKDTLMISRTPEVTCVVSGYNPYDFPIVKFKWYVDGVEVHNAKTNPRDENSYNTDRVVSKLTVLHQDWLSGKEYKCKVSAREGGSSGEWYYNLWGPIECTISKAK

SEQ ID NO: 22 - protein, 114 aa, synthetic construct
PSVLCLPPKPKDTLMISRTPEVTCVVSGYNPYDFPIVNFKWYVDGVEVHNAKTKPRDENSYNTDRVVSKLTVLHQDWLNGKEYKCKVSAREGGSSGDWYYDLWGPIECTISKAK

SEQ ID NO: 23 - protein, 114 aa, synthetic construct
PSVLCLPPEPKDTLMISRTPEVTCVVSGYNPYDFPIVKFKWYVDGVEVHNAKTKPRDENSYNTDRVVSKLIVLHQDWLNGKEYKCKVSAREGGSSGEWYYDLWGPIECTISIAK

SEQ ID NO: 24 - protein, 114 aa, synthetic construct
PSVLCLPPKPKDTLVISRTPEVTCVVSGYNPYDFPIIKFKWYVDGVEVDNAKVKPRDENSYNTDSVVSKLTVLHQDWLNGKEYKCKVSARVGGSSGEWYYDLWGPIECTISKAK

SEQ ID NO: 25 - protein, 114 aa, synthetic construct
PSVLCLPPKPKDTLVISRTPEVTCVVSGYNPYDFPIIKFKWYVDGVEVDNAKVKPRDENSYNTDSVVSKLTVLHQDWLNGKEYKCKVSAREGGSSGEWYYDLWGPIECTISIKS

SEQ ID NO: 26 - protein, 114 aa, synthetic construct
PSVHCHPPKPKDTLVISRTPEVTCVVSGYNPYDFPIIKFKWYVDGVEVDNAKVKPRDENSYNTDSVVSKLTVKHQDWLNGKEYKCKVSAREGGSSGEWYYDLWGPIECTISKAK

SEQ ID NO: 27 - protein, 114 aa, synthetic construct
PSVHCHPPKPKDTLVISRTPEVTCVVSGYNPYDFPIIKFKWYVDGVEVDNAKVKPRDENSYNTDSVVSKLTVKHQDWLNGKEYKCKVSAREGGSSGEWYYDLWGPIECTISIKS

SEQ ID NO: 28 - protein, 114 aa, synthetic construct
PSVLCLPPKSNDALVISRTPEVTCVVSGYNPYDFPIIKFKWYVDGVEVDNAKVKPRDENSYNTDSVVSKLTILHQDWLNGKEYKCKVSAREGGSSGEWYYDLWGPIECTISKAK

SEQ ID NO: 29 - protein, 114 aa, synthetic construct
PSVLCLPPKSNDALVISRTPEVTCVVSGYNPYDFPIIKFKWYVDGVEVDNAKVKPRDENSYNTDSVVSKLTILHQDWLNGKEYKCKVSAREGGSSGEWYYDLWGPIECTISIKS

SEQ ID NO: 30 - protein, 114 aa, synthetic construct
PSVHCHPPKSNDALVISRTPEVTCVVSGYNPYDFPIIKFKWYVDGVEVDNAKVKPRDENSYNTDSVVSKLTIKHQDWLNGKEYKCKVSAREGGSSGEWYYDLWGPIECTISKAK

SEQ ID NO: 31 - protein, 114 aa, synthetic construct
PSVHCHPPKSNDALVISRTPEVTCVVSGYNPYDFPIIKFKWYVDGVEVDNAKVKPRDENSYNTDSVVSKLTIKHQDWLNGKEYKCKVSAREGGSSGEWYYDLWGPIECTISIKS

SEQ ID NO: 32 - protein, 114 aa, synthetic construct
PSVFLFPPKPKDTLMISRTPEVTCVVVGYNPYDFPIIKFNWYVDGVEVHNAKTKPRDENSYNTDSVVSVLTVLHQDWLNGKEYKCKVSAREGGSSGEWYYDLWGPIEKTISKAK

SEQ ID NO: 33 - protein, 114 aa, synthetic construct
PSVFCFPPKPKDTLMISRTPEVTCVVVGYNPYDFPIIQFNWYVDGVEVHNAKTKPRDENSYNTDSVVSVLTVVHQDWLNGKEYKCKVSAREGGSSGEWYYDLWGPIECTISKTK

SEQ ID NO: 34 - protein, 114 aa, synthetic construct
PSVFCFPPKPKDTLMISRTPEVTCVVVGYNPYDFPIIQFKWYVDGVEVHNAKTKPRDENSYNTDSVVSVLTVLHQDWLNGKEYKCKVSAREGGSSGEWYYDLWGPIECTISKTK

SEQ ID NO: 35 - protein, 114 aa, synthetic construct
PSVFCFPPKPKDTLMISRTPEVTCVVVGYNPYDFPIIQFNWYVDGVEVHNAKTKPRDENSYNTDSVVSVLTVLHQDWLNGKEYKCKVSAREGGSSGEWYYDLWGSIECTISKAK

SEQ ID NO: 36 - protein, 153 aa, synthetic construct
PSVLCLPPKPKDTLVISRTPEVTCVVSGYNPYDFPIIKFKWYVDGVEVDNAKVKPRDENSYNTDSVVSKLTVLHQDWLNGKEYKCKVSAREGGSSGEWYYDLWGPIECTISKAKGGSTIDQWLLKNAKEDAIAELKKAGITSDFYFNAINKAK

SEQ ID NO: 37 - protein, 130 aa, synthetic construct
PSVLCLPPKPKDTLVISRTPEVTCVVSGYNPYDFPIIKFKWYVDGVEVDNAKVKPRDENSYNTDSVVSKLTVLHQDWLNGKEYKCKVSAREGGSSGEWYYDLWGPIECTISKAKQRFVTGHFGGLHPANG

SEQ ID NO: 38 - protein, 251 aa, synthetic construct
PSVLCLPPKPKDTLVISRTPEVTCVVSGYNPYDFPIIKFKWYVDGVEVDNAKVKPRDENSYNTDSVVSKLTVLHQDWLNGKEYKCKVSAREGGSSGEWYYDLWGPIECTISKAKGGSGGSGGSGGSGGSGGSGGSGAVQLVESGGGLVQPGNSLRLSCAASGFTFRSFGMSWVRQAPGKEPEWVSSISGSGSDTLYADSVKGRFTISRDNAKTTLYLQMNSLKPEDTAVYYCTIGGSLSRSSQGTQVTVSS

SEQ ID NO: 39 - DNA, 30 bp, synthetic construct
  source 1..30: mol_type = other DNA
ggttataacccctacgactttcctattatt

SEQ ID NO: 40 - DNA, 27 bp, synthetic construct
  source 1..27: mol_type = other DNA
gatgagaactcttacaacaccgatagt

SEQ ID NO: 41 - DNA, 48 bp, synthetic construct
  source 1..48: mol_type = other DNA
gcgcgagagggtgggtcctcgggggagtggtactacgatctgtggggc

SEQ ID NO: 42 - DNA, 342 bp, synthetic construct
  source 1..342: mol_type = other DNA
ccgtcagtcttgtgcctgcccccaaaacccaaggacaccctcgtgatctcccggacccctgaggtcacatgcgtggtgtctggttataacccctacgactttcctattattaagttcaaatggtacgtggacggcgtggaggtggataatgccaaggtaaagccgcgggatgagaactcttacaacaccgatagtgtggtcagcaaactcaccgtcctgcaccaggactggctgaatggcaaggagtacaagtgcaaggtcagtgcgcgagagggtgggtcctcgggggagtggtactacgatctgtggggccccatcgaatgcaccatctccaaagccaaa